European Patent Specification EP 3 512 886 B1, published June 11, 2025. Title: Antigen binding protein against HER3. Applicant: Universität Stuttgart. The sequence listing filed with the application follows.

SEQUENCE LISTING (35 sequences)

SEQ ID NO: 1 - protein, 1342 aa, Homo sapiens
MRANDALQVLGLLFSLARGSEVGNSQAVCPGTLNGLSVTGDAENQYQTLYKLYERCEVVMGNLEIVLTGHNADLSFLQWIREVTGYVLVAMNEFSTLPLPNLRVVRGTQVYDGKFAIFVMLNYNTNSSHALRQLRLTQLTEILSGGVYIEKNDKLCHMDTIDWRDIVRDRDAEIVVKDNGRSCPPCHEVCKGRCWGPGSEDCQTLTKTICAPQCNGHCFGPNPNQCCHDECAGGCSGPQDTDCFACRHFNDSGACVPRCPQPLVYNKLTFQLEPNPHTKYQYGGVCVASCPHNFVVDQTSCVRACPPDKMEVDKNGLKMCEPCGGLCPKACEGTGSGSRFQTVDSSNIDGFVNCTKILGNLDFLITGLNGDPWHKIPALDPEKLNVFRTVREITGYLNIQSWPPHMHNFSVFSNLTTIGGRSLYNRGFSLLIMKNLNVTSLGFRSLKEISAGRIYISANRQLCYHHSLNWTKVLRGPTEERLDIKHNRPRRDCVAEGKVCDPLCSSGGCWGPGPGQCLSCRNYSRGGVCVTHCNFLNGEPREFAHEAECFSCHPECQPMEGTATCNGSGSDTCAQCAHFRDGPHCVSSCPHGVLGAKGPIYKYPDVQNECRPCHENCTQGCKGPELQDCLGQTLVLIGKTHLTMALTVIAGLVVIFMMLGGTFLYWRGRRIQNKRAMRRYLERGESIEPLDPSEKANKVLARIFKETELRKLKVLGSGVFGTVHKGVWIPEGESIKIPVCIKVIEDKSGRQSFQAVTDHMLAIGSLDHAHIVRLLGLCPGSSLQLVTQYLPLGSLLDHVRQHRGALGPQLLLNWGVQIAKGMYYLEEHGMVHRNLAARNVLLKSPSQVQVADFGVADLLPPDDKQLLYSEAKTPIKWMALESIHFGKYTHQSDVWSYGVTVWELMTFGAEPYAGLRLAEVPDLLEKGERLAQPQICTIDVYMVMVKCWMIDENIRPTFKELANEFTRMARDPPRYLVIKRESGPGIAPGPEPHGLTNKKLEEVELEPELDLDLDLEAEEDNLATTTLGSALSLPVGTLNRPRGSQSLLSPSSGYMPMNQGNLGESCQESAVSGSSERCPRPVSLHPMPRGCLASESSEGHVTGSEAELQEKVSMCRSRSRSRSPRPRGDSAYHSQRHSLLTPVTPLSPPGLEEEDVNGYVMPDTHLKGTPSSREGTLSSVGLSSVLGTEEEDEDEEYEYMNRRRRHSPPHPPRPSSLEELGYEYMDVGSDLSASLGSTQSCPLHPVPIMPTAGTTPDEDYEYMNRQRDGGGPGGDYAAMGACPASEQGYEEMRAFQGPGHQAPHVHYARLKTLRSLEATDSAFDNPDYWHSRLFPKANAQRT

SEQ ID NO: 2 - protein, 123 aa, Artificial Sequence
  variable domain heavy chain of 3-43
QVQLQQSGPGLVKPSQTLSLTCAISGDSVSSNRAAWNWIRQSPSRGLEWLGRTYYRSKWYNDYAQSLKSRITINPDTPKNQFSLQLNSVTPEDTAVYYCARDGQLGLDALDIWGQGTMVTVSS

SEQ ID NO: 3 - protein, 109 aa, Artificial Sequence
  variable domain light chain of 3-43
QAGLTQPPAVSVAPGQTASITCGRDNIGSRSVHWYQQKPGQAPVLVVYDDSDRPAGIPERFSGSNYENTATLTISRVEAGDEADYYCQVWGITSDHVVFGGGTKLTVLG

SEQ ID NO: 4 - protein, 473 aa, Artificial Sequence
  IgK leader - IgG 3-43 HC
METDTLLLWVLLLWVPGSTGQVQLQQSGPGLVKPSQTLSLTCAISGDSVSSNRAAWNWIRQSPSRGLEWLGRTYYRSKWYNDYAQSLKSRITINPDTPKNQFSLQLNSVTPEDTAVYYCARDGQLGLDALDIWGQGTMVTVSSASTKGPSVFPLAPSSKSTSGGTAALGCLVKDYFPEPVTVSWNSGALTSGVHTFPAVLQSSGLYSLSSVVTVPSSSLGTQTYICNVNHKPSNTKVDKKVEPKSCDKTHTCPPCPAPELLGGPDVFLFPPKPKDTLMISRTPEVTCVVVDVSHEDPEVKFNWYVDGVEVHNAKTKPREEQYNSTYRVVSVLTVLHQDWLNGKEYKCKVSNKALPAPEEKTISKAKGQPREPQVYTLPPSRDELTKNQVSLTCLVKGFYPSDIAVEWESNGQPENNYKTTPPVLDSDGSFFLYSKLTVDKSRWQQGNVFSCSVMHEALHNHYTQKSLSLSPGK

SEQ ID NO: 5 - protein, 235 aa, Artificial Sequence
  IgK leader - IgG 3-43 LC
METDTLLLWVLLLWVPGSTGQAGLTQPPAVSVAPGQTASITCGRDNIGSRSVHWYQQKPGQAPVLVVYDDSDRPAGIPERFSGSNYENTATLTISRVEAGDEADYYCQVWGITSDHVVFGGGTKLTVLCGQPKAAPSVTLFPPSSEELQANKATLVCLISDFYPGAVTVAWKADSSPVKAGVETTTPSKQSNNKYAASSYLSLTPEQWKSHRSYSCQVTHEGSTVEKTVAPTECS

SEQ ID NO: 6 - protein, 247 aa, Artificial Sequence
  scFv 3-43
QVQLQQSGPGLVKPSQTLSLTCAISGDSVSSNRAAWNWIRQSPSRGLEWLGRTYYRSKWYNDYAQSLKSRITINPDTPKNQFSLQLNSVTPEDTAVYYCARDGQLGLDALDIWGQGTMVTVSSGGGGSGGGGSGGGGSQAGLTQPPAVSVAPGQTASITCGRDNIGSRSVHWYQQKPGQAPVLVVYDDSDRPAGIPERFSGSNYENTATLTISRVEAGDEADYYCQVWGITSDHVVFGGGTKLTVLG

SEQ ID NO: 7 - protein, 310 aa, Artificial Sequence
  PelB leader - scFv 3-43 - c-myc - his
MKYLLPTAAAGLLLLAAQPAMAQVQLQQSGPGLVKPSQTLSLTCAISGDSVSSNRAAWNWIRQSPSRGLEWLGRTYYRSKWYNDYAQSLKSRITINPDTPKNQFSLQLNSVTPEDTAVYYCARDGQLGLDALDIWGQGTMVTVSSGSASAPKLEEGEFSEARVQAGLTQPPAVSVAPGQTASITCGRDNIGSRSVHWYQQKPGQAPVLVVYDDSDRPAGIPERFSGSNYENTATLTISRVEAGDEADYYCQVWGITSDHVVFGGGTKLTVLGQPKAAPSVTLFPPSSAAAEQKLISEEDLNGAAHHHHHH

SEQ ID NO: 8 - protein, 738 aa, Artificial Sequence
  IgK leader - scDb hu225x3-43-Fc
METDTLLLWVLLLWVPGSTGEVQLVESGGGLVQPGGSLRLSCAASGFSLTNYGVHWVRQAPGKGLEWLGVIWSGGNTDYNTPFTSRFTISRDNSKNTLYLQMNSLRAEDTAVYYCARALTYYDYEFAYWGQGTTVTVSSGGGGSQAGLTQPPAVSVAPGQTASITCGRDNIGSRSVHWYQQKPGQAPVLVVYDDSDRPAGIPERFSGSNYENTATLTISRVEAGDEADYYCQVWGITSDHVVFGGGTKLTVLGGGGSGGRASGGGGSQVQLQQSGPGLVKPSQTLSLTCAISGDSVSSNRAAWNWIRQSPSRGLEWLGRTYYRSKWYNDYAQSLKSRITINPDTPKNQFSLQLNSVTPEDTAVYYCARDGQLGLDALDIWGQGTMVTVSSGGGGSDIQLTQSPSFLSASVGDRVTITCRASQSIGTNIHWYQQKPGKAPKLLIKYASESISGVPSRFSGSGSGTEFTLTISSLQPEDFATYYCQQNNNWPTTFGAGTKLEIKRAAAGGSGGDKTHTCPPCPAPELLGGPSVFLFPPKPKDTLMISRTPEVTCVVVDVSHEDPEVKFNWYVDGVEVHNAKTKPREEQYNSTYRVVSVLTVLHQDWLNGKEYKCKVSNKALPAPIEKTISKAKGQPREPQVYTLPPSRDELTKNQVSLTCLVKGFYPSDIAVEWESNGQPENNYKTTPPVLDSDGSFFLYSKLTVDKSRWQQGNVFSCSVMHEALHNHYTQKSLSLSPGK

SEQ ID NO: 9 - protein, 744 aa, Artificial Sequence
  IgK leader 2-35 x 3-43 scDb-Fc
METDTLLLWVLLLWVPGSTGQMQLVQSGAEVKKPGESLKISCKGSGYSFTSYWIGWVRQMPGKGLEWMGIIYPGDSDTRYSPSFQGQVTISADKSISTAYLQWSSLKASDTAMYYCARLGRSGSYYNYGMDVWGQGTTVTVSSGGGGSQAGLTQPPAVSVAPGQTASITCGRDNIGSRSVHWYQQKPGQAPVLVVYDDSDRPAGIPERFSGSNYENTATLTISRVEAGDEADYYCQVWGITSDHVVFGGGTKLTVLGGGGSGGRASGGGGSQVQLQQSGPGLVKPSQTLSLTCAISGDSVSSNRAAWNWIRQSPSRGLEWLGRTYYRSKWYNDYAQSLKSRITINPDTPKNQFSLQLNSVTPEDTAVYYCARDGQLGLDALDIWGQGTMVTVSSGGGGSQAVVTQEPSFSVSPGGTVTLTCGLSSGSVSSSYYPSWYQQTSGQPPRTLIYSTDTRSSGVPDRFSGSILGDKAALTITGAQADDESDYYCMLYMGSGISVFGGGTKLAVLAAAGGSGGDKTHTCPPCPAPELLGGPSVFLFPPKPKDTLMISRTPEVTCVVVDVSHEDPEVKFNWYVDGVEVHNAKTKPREEQYNSTYRVVSVLTVLHQDWLNGKEYKCKVSNKALPAPIEKTISKAKGQPREPQVYTLPPSRDELTKNQVSLTCLVKGFYPSDIAVEWESNGQPENNYKTTPPVLDSDGSFFLYSKLTVDKSRWQQGNVFSCSVMHEALHNHYTQKSLSLSPGK

SEQ ID NO: 10 - protein, 744 aa, Artificial Sequence
  IgK leader - scDb 4D5x3-43-LL-Fc
METDTLLLWVLLLWVPGSTGEVQLVESGGGLVQPGGSLRLSCAASGFNIKDTYIHWVRQAPGKGLEWVARIYPTNGYTRYADSVKGRFTISADTSKNTAYLQMNSLRAEDTAVYYCSRWGGDGFYAMDYWGQGTLVTVSSGGGGSQAGLTQPPAVSVAPGQTASITCGRDNIGSRSVHWYQQKPGQAPVLVVYDDSDRPAGIPERFSGSNYENTATLTISRVEAGDEADYYCQVWGITSDHVVFGGGTKLTVLGGGGSGGRASGGGGSGGGGSQVQLQQSGPGLVKPSQTLSLTCAISGDSVSSNRAAWNWIRQSPSRGLEWLGRTYYRSKWYNDYAQSLKSRITINPDTPKNQFSLQLNSVTPEDTAVYYCARDGQLGLDALDIWGQGTMVTVSSGGGGSDIQMTQSPSSLSASVGDRVTITCRASQDVNTAVAWYQQKPGKAPKLLIYSASFLYSGVPSRFSGSRSGTDFTLTISSLQPEDFATYYCQQHYTTPPTFGQGTKVEIKRAAAGGSGGDKTHTCPPCPAPELLGGPSVFLFPPKPKDTLMISRTPEVTCVVVDVSHEDPEVKFNWYVDGVEVHNAKTKPREEQYNSTYRVVSVLTVLHQDWLNGKEYKCKVSNKALPAPIEKTISKAKGQPREPQVYTLPPSRDELTKNQVSLTCLVKGFYPSDIAVEWESNGQPENNYKTTPPVLDSDGSFFLYSKLTVDKSRWQQGNVFSCSVMHEALHNHYTQKSLSLSPGK

SEQ ID NO: 11 - protein, 1020 aa, Artificial Sequence
  IgK leader - FLAG - linker - scFv3-43-Fc-scTRAIL
METDTLLLWVLLLWVPGSTGDYKDDDDKGGGGSGTQVQLQQSGPGLVKPSQTLSLTCAISGDSVSSNRAAWNWIRQSPSRGLEWLGRTYYRSKWYNDYAQSLKSRITINPDTPKNQFSLQLNSVTPEDTAVYYCARDGQLGLDALDIWGQGTMVTVSSGGGGSGGGGSGGGGSQAGLTQPPAVSVAPGQTASITCGRDNIGSRSVHWYQQKPGQAPVLVVYDDSDRPAGIPERFSGSNYENTATLTISRVEAGDEADYYCQVWGITSDHVVFGGGTKLTVLAAAGGSGGDKTHTCPPCPAPELLGGPSVFLFPPKPKDTLMISRTPEVTCVVVDVSHEDPEVKFNWYVDGVEVHNAKTKPREEQYNSTYRVVSVLTVLHQDWLNGKEYKCKVSNKALPAPIEKTISKAKGQPREPQVYTLPPSRDELTKNQVSLTCLVKGFYPSDIAVEWESNGQPENNYKTTPPVLDSDGSFFLYSKLTVDKSRWQQGNVFSCSVMHEALHNHYTQKSLSLSPGQGGSGGGSSGGGPQRVAAHITGTRGRSNTLSSPNSKNEKALGRKINSWESSRSGHSFLSNLHLRNGELVIHEKGFYYIYSQTYFRFQEEIKENTKNDKQMVQYIYKYTSYPDPILLMKSARNSCWSKDAEYGLYSIYQGGIFELKENDRIFVSVTNEHLIDMDHEASFFGAFLVGGGPQRVAAHITGTRGRSNTLSSPNSKNEKALGRKINSWESSRSGHSFLSNLHLRNGELVIHEKGFYYIYSQTYFRFQEEIKENTKNDKQMVQYIYKYTSYPDPILLMKSARNSCWSKDAEYGLYSIYQGGIFELKENDRIFVSVTNEHLIDMDHEASFFGAFLVGGGPQRVAAHITGTRGRSNTLSSPNSKNEKALGRKINSWESSRSGHSFLSNLHLRNGELVIHEKGFYYIYSQTYFRFQEEIKENTKNDKQMVQYIYKYTSYPDPILLMKSARNSCWSKDAEYGLYSIYQGGIFELKENDRIFVSVTNEHLIDMDHEASFFGAFLVG

SEQ ID NO: 12 - protein, 515 aa, Artificial Sequence
  IgK leader - scDb 3-43xCD3 - His
METDTLLLWVLLLWVPGSTGQVQLQQSGPGLVKPSQTLSLTCAISGDSVSSNRAAWNWIRQSPSRGLEWLGRTYYRSKWYNDYAQSLKSRITINPDTPKNQFSLQLNSVTPEDTAVYYCARDGQLGLDALDIWGQGTMVTVSSGGGGSDIQMTQSPSSLSASVGDRVTITCRASQDIRNYLNWYQQKPGKAPKLLIYYTSRLHSGVPSRFSGSGSGTDFTFTISSLQPEDIATYYCQQGNTLPWTFGQGTKLEIKRGGGGSGGGGSGGGGSQVQLVQSGAEVKKPGSSVKVSCKASGGTFSGYTMNWVRQAPGQGLEWMGLINPYKGVSTYNGKFKDRVTITADKSTSTAYMELSSLRSEDTAVYYCARSGYYGDSDWYFDVWGQGTLVTVSSGGGGSQAGLTQPPAVSVAPGQTASITCGRDNIGSRSVHWYQQKPGQAPVLVVYDDSDRPAGIPERFSGSNYENTATLTISRVEAGDEADYYCQVWGITSDHVVFGGGTKLTVLAAAHHHHHH

SEQ ID NO: 13 - protein, 776 aa, Artificial Sequence
  IgK leader - scDb 3-43xCD3-scFv 3-43 - His
METDTLLLWVLLLWVPGSTGQVQLQQSGPGLVKPSQTLSLTCAISGDSVSSNRAAWNWIRQSPSRGLEWLGRTYYRSKWYNDYAQSLKSRITINPDTPKNQFSLQLNSVTPEDTAVYYCARDGQLGLDALDIWGQGTMVTVSSGGGGSDIQMTQSPSSLSASVGDRVTITCRASQDIRNYLNWYQQKPGKAPKLLIYYTSRLHSGVPSRFSGSGSGTDFTFTISSLQPEDIATYYCQQGNTLPWTFGQGTKLEIKRGGGGSGGGGSGGGGSQVQLVQSGAEVKKPGSSVKVSCKASGGTFSGYTMNWVRQAPGQGLEWMGLINPYKGVSTYNGKFKDRVTITADKSTSTAYMELSSLRSEDTAVYYCARSGYYGDSDWYFDVWGQGTLVTVSSGGGGSQAGLTQPPAVSVAPGQTASITCGRDNIGSRSVHWYQQKPGQAPVLVVYDDSDRPAGIPERFSGSNYENTATLTISRVEAGDEADYYCQVWGITSDHVVFGGGTKLTVLAAAGGSGGGGSGGGTQVQLQQSGPGLVKPSQTLSLTCAISGDSVSSNRAAWNWIRQSPSRGLEWLGRTYYRSKWYNDYAQSLKSRITINPDTPKNQFSLQLNSVTPEDTAVYYCARDGQLGLDALDIWGQGTMVTVSSGGGGSGGGGSGGGGSQAGLTQPPAVSVAPGQTASITCGRDNIGSRSVHWYQQKPGQAPVLVVYDDSDRPAGIPERFSGSNYENTATLTISRVEAGDEADYYCQVWGITSDHVVFGGGTKLTVLGSLHHHHHH

SEQ ID NO: 14 - protein, 5 aa, Artificial Sequence
  peptide linker 1
GGGGS

SEQ ID NO: 15 - protein, 10 aa, Artificial Sequence
  peptide linker 2
GGGGSGGGGS

SEQ ID NO: 16 - protein, 15 aa, Artificial Sequence
  peptide linker 3
GGGGSGGGGSGGGGS

SEQ ID NO: 17 - protein, 8 aa, Artificial Sequence
  peptide linker 4
GSLGGSGG

SEQ ID NO: 18 - protein, 8 aa, Artificial Sequence
  peptide linker 5
GGGSGGGT

SEQ ID NO: 19 - protein, 10 aa, Artificial Sequence
  peptide linker 6
GGGSGGGTGS

SEQ ID NO: 20 - protein, 12 aa, Artificial Sequence
  peptide linker 7
GGGSGGGTGSGG

SEQ ID NO: 21 - protein, 20 aa, Artificial Sequence
  peptide linker 8
GGGGSGGRASGGGGSGGGGS

SEQ ID NO: 22 - protein, 8 aa, Artificial Sequence
  peptide linker 9
GGGSGGGS

SEQ ID NO: 23 - protein, 5 aa, Artificial Sequence
  peptide linker 10
EFTRG

SEQ ID NO: 24 - protein, 3 aa, Artificial Sequence
  peptide linker 11
AAA

SEQ ID NO: 25 - protein, 8 aa, Artificial Sequence
  FLAG-tag
DYKDDDDK

SEQ ID NO: 26 - protein, 6 aa, Artificial Sequence
  His-tag
HHHHHH

SEQ ID NO: 27 - protein, 10 aa, Artificial Sequence
  Myc-tag
EQKLISEEDL

SEQ ID NO: 28 - protein, 22 aa, Artificial Sequence
  PelB leader sequence
MKYLLPTAAAGLLLLAAQPAMA

SEQ ID NO: 29 - protein, 20 aa, Artificial Sequence
  IgK leader sequence
METDTLLLWVLLLWVPGSTG

SEQ ID NO: 30 - protein, 20 aa, Artificial Sequence
  IL-2 leader sequence
MYRMQLLSCIALSLALVTNS

SEQ ID NO: 31 - protein, 342 aa, Artificial Sequence
  VH3-43xVLhu225-CL
QVQLQQSGPGLVKPSQTLSLTCAISGDSVSSNRAAWNWIRQSPSRGLEWLGRTYYRSKWYNDYAQSLKSRITINPDTPKNQFSLQLNSVTPEDTAVYYCARDGQLGLDALDIWGQGTMVTVSSGGGGSDIQLTQSPSFLSASVGDRVTITCRASQSIGTNIHWYQQKPGKAPKLLIKYASESISGVPSRFSGSGSGTEFTLTISSLQPEDFATYYCQQNNNWPTTFGAGTKLEIKRTVAAPSVFIFPPSDEQLKSGTASVVCLLNNFYPREAKVQWKVDNALQSGNSQESVTEQDSKDSTYSLSSTLTLSKADYEKHKVYACEVTHQGLSSPVTKSFNRGEC

SEQ ID NO: 32 - protein, 561 aa, Artificial Sequence
  VHhu225xVLhu3-43-CH1-CH2-CH3
EVQLVESGGGLVQPGGSLRLSCAASGFSLTNYGVHWVRQAPGKGLEWLGVIWSGGNTDYNTPFTSRFTISRDNSKNTLYLQMNSLRAEDTAVYYCARALTYYDYEFAYWGQGTTVTVSSGGGGSQAGLTQPPAVSVAPGQTASITCGRDNIGSRSVHWYQQKPGQAPVLVVYDDSDRPAGIPERFSGSNYENTATLTISRVEAGDEADYYCQVWGITSDHVVFGGGTKLTVLASTKGPSVFPLAPSSKSTSGGTAALGCLVKDYFPEPVTVSWNSGALTSGVHTFPAVLQSSGLYSLSSVVTVPSSSLGTQTYICNVNHKPSNTKVDKKVEPKSCDKTHTCPPCPAPPVAGPSVFLFPPKPKDTLMISRTPEVTCVVVDVSHEDPEVKFNWYVDGVEVHNAKTKPREEQYNSTYRVVSVLTVLHQDWLNGKEYKCKVSNKGLPSSIEKTISKAKGQPREPQVYTLPPSRDELTKNQVSLTCLVKGFYPSDIAVEWESNGQPENNYKTTPPVLDSDGSFFLYSKLTVDKSRWQQGNVFSCSVMHEALHNHYTQKSLSLSPGK

SEQ ID NO: 33 - protein, 738 aa, Artificial Sequence
  scDbhu225x3-43-Fc(GGGGS)
METDTLLLWVLLLWVPGSTGEVQLVESGGGLVQPGGSLRLSCAASGFSLTNYGVHWVRQAPGKGLEWLGVIWSGGNTDYNTPFTSRFTISRDNSKNTLYLQMNSLRAEDTAVYYCARALTYYDYEFAYWGQGTTVTVSSGGGGSQAGLTQPPAVSVAPGQTASITCGRDNIGSRSVHWYQQKPGQAPVLVVYDDSDRPAGIPERFSGSNYENTATLTISRVEAGDEADYYCQVWGITSDHVVFGGGTKLTVLGGGGSGGGGSGGGGSQVQLQQSGPGLVKPSQTLSLTCAISGDSVSSNRAAWNWIRQSPSRGLEWLGRTYYRSKWYNDYAQSLKSRITINPDTPKNQFSLQLNSVTPEDTAVYYCARDGQLGLDALDIWGQGTMVTVSSGGGGSDIQLTQSPSFLSASVGDRVTITCRASQSIGTNIHWYQQKPGKAPKLLIKYASESISGVPSRFSGSGSGTEFTLTISSLQPEDFATYYCQQNNNWPTTFGAGTKLEIKRAAAGGSGGDKTHTCPPCPAPELLGGPSVFLFPPKPKDTLMISRTPEVTCVVVDVSHEDPEVKFNWYVDGVEVHNAKTKPREEQYNSTYRVVSVLTVLHQDWLNGKEYKCKVSNKALPAPIEKTISKAKGQPREPQVYTLPPSRDELTKNQVSLTCLVKGFYPSDIAVEWESNGQPENNYKTTPPVLDSDGSFFLYSKLTVDKSRWQQGNVFSCSVMHEALHNHYTQKSLSLSPGK

SEQ ID NO: 34 - protein, 519 aa, Artificial Sequence
  scDb4D5x3-43-LL
METDTLLLWVLLLWVPGSTGDAAQPAMAEVQLVESGGGLVQPGGSLRLSCAASGFNIKDTYIHWVRQAPGKGLEWVARIYPTNGYTRYADSVKGRFTISADTSKNTAYLQMNSLRAEDTAVYYCSRWGGDGFYAMDYWGQGTLVTVSSGGGGSQAGLTQPPAVSVAPGQTASITCGRDNIGSRSVHWYQQKPGQAPVLVVYDDSDRPAGIPERFSGSNYENTATLTISRVEAGDEADYYCQVWGITSDHVVFGGGTKLTVLGGGGSGGRASGGGGSGGGGSQVQLQQSGPGLVKPSQTLSLTCAISGDSVSSNRAAWNWIRQSPSRGLEWLGRTYYRSKWYNDYAQSLKSRITINPDTPKNQFSLQLNSVTPEDTAVYYCARDGQLGLDALDIWGQGTMVTVSSGGGGSDIQMTQSPSSLSASVGDRVTITCRASQDVNTAVAWYQQKPGKAPKLLIYSASFLYSGVPSRFSGSRSGTDFTLTISSLQPEDFATYYCQQHYTTPPTFGQGTKVEIKRAA

SEQ ID NO: 35 - protein, 770 aa, Artificial Sequence
  scFv3-43-scDb3-43xhuU3-scFv3-43
METDTLLLWVLLLWVPGSTGQVQLQQSGPGLVKPSQTLSLTCAISGDSVSSNRAAWNWIRQSPSRGLEWLGRTYYRSKWYNDYAQSLKSRITINPDTPKNQFSLQLNSVTPEDTAVYYCARDGQLGLDALDIWGQGTMVTVSSGGGGSDIQMTQSPSSLSASVGDRVTITCRASQDIRNYLNWYQQKPGKAPKLLIYYTSRLHSGVPSRFSGSGSGTDFTFTISSLQPEDIATYYCQQGNTLPWTFGQGTKLEIKRGGGGSGGGGSGGGGSQVQLVQSGAEVKKPGSSVKVSCKASGGTFSGYTMNWVRQAPGQGLEWMGLINPYKGVSTYNGKFKDRVTITADKSTSTAYMELSSLRSEDTAVYYCARSGYYGDSDWYFDVWGQGTLVTVSSGGGGSQAGLTQPPAVSVAPGQTASITCGRDNIGSRSVHWYQQKPGQAPVLVVYDDSDRPAGIPERFSGSNYENTATLTISRVEAGDEADYYCQVWGITSDHVVFGGGTKLTVLAAAGGSGGGGSGGGTQVQLQQSGPGLVKPSQTLSLTCAISGDSVSSNRAAWNWIRQSPSRGLEWLGRTYYRSKWYNDYAQSLKSRITINPDTPKNQFSLQLNSVTPEDTAVYYCARDGQLGLDALDIWGQGTMVTVSSGGGGSGGGGSGGGGSQAGLTQPPAVSVAPGQTASITCGRDNIGSRSVHWYQQKPGQAPVLVVYDDSDRPAGIPERFSGSNYENTATLTISRVEAGDEADYYCQVWGITSDHVVFGGGTKLTVLGSL